European Patent Application EP 4 729 525 A1, published April 22, 2026. Title: Newly synthesized boron-nitrogen heterocycles and their conjugates with pharmaceutically utilizable substances. Applicant: Julius-Maximilians-Universitaet Wuerzburg. Application EP. The sequence listing filed with the application follows.

SEQUENCE LISTING (1 sequence)

SEQ ID NO: 1 - protein, 518 aa, Aplysia punctata
MDGVSRNRRQCNREVCGSTYDVAVVGAGPGGANSAYMLRDSGLDIAVFEYSDRVGGRLFTYQLPNTPDVNLEIGGMRFIEGAMHRLWRVISELGLTPKVFKEGFGKEGRQRFYLRGQSLTKKQVKSGDVPYDLSPEEKENQGNLVEYYLEKLTGLQLNGEPLKREVALKLTVPDGRFLYDLSFDEAMDLVASPEGKEFTRDTHVFTGEVTLDASAVSLFDDHLGEDYYGSEIYTLKEGLSSVPQGLLQAFLDAADSNEFYPNSHLKALRRKTNGQYVLYFEPTTSKDGQTTINYLEPLQVVCAQRVILAMPVYALNQLDWNQLRNDRATQAYAAVRPIPASKVFMTFDQPWWLENERKSWVTKSDALFSQMYDWQKSEASGDYILIASYADGLKAQYLRELKNQGEDIPGSDPGYNQVTEPLKDTILDHLTEAYGVERDSIPEPVTAASQFWTDYPFGCGWITWRAGFHFDDVISTMRRPSLKDEVYVVGADYSWGLISSWIEGALETSENVINDYFL